European Patent Specification EP 3 696 264 B1, published June 28, 2023. Title: COMPOSITIONS AND METHODS COMPRISING A LIPOLYTIC ENZYME VARIANT. Applicant: DANISCO US INC. GRAYCAR, Thomas P. POULOSE, Ayrookaran J. ESTELL, David A. Application Not assigned. The sequence listing filed with the application follows.

SEQUENCE LISTING (3 sequences)

SEQ ID NO: 1 - protein, 269 aa, Thermomyces lanuginosa [sequence omitted]

SEQ ID NO: 2 - protein, 269 aa, Thermomyces lanuginosa
  misc_feature: sequence of the reference lipolytic enzyme, which is a variant from Thermomyces lanuginosa (TLL)
EVSQDLFNQFNLFAQYSAAAYCGKNNDAPAGTNITCTGNACPEVEKADATFLYSFEDSGVGDVTGFLALDNTNKLIVLSFRGSRSIENWIGNLNFDLKEINDICSGCRGHDGFTSSWRSVADTLRQKVEDAVREHPDYRVVFTGHSLGGALATVAGADLRGNGYDIDVFSYGAPRVGNRAFAEFLTVQTGGTLYRITHTNDIVPRLPPREFGYSHSSPEYWIKSGTLVPVRRRDIVKIEGIDATGGNNQPNIPDIPAHLWYFGLIGTCL

SEQ ID NO: 3 - DNA, 834 bp, Artificial Sequence
  Nucleotide sequence of the synthetic TLL gene
gctagcgcagctggcaaagaagttagccaagatctgttcaaccaattcaaccttttcgctcaatactctgcagctgcttactgcggaaagaacaacgatgcacctgctggtactaacatcacttgcacaggtaacgcatgtcctgaagtagaaaaagctgatgctacatttctttactcttttgaagatagcggcgtcggcgatgttaccggtttcttagctctggataacacaaacaaacttatcgtccttagcttcagaggctctcgctcaatcgaaaactggatcggtaaccttaattttgacttgaaagaaatcaacgatatctgctctggttgccgtggccatgacggattcacatcatcttggagaagcgtcgcagacacgcttcgccaaaaagtagaagatgccgtacgcgaacacccagattacagagtagttttcacaggtcactctcttggcggagctttagcaacagtagcaggcgctgatctccgcggtaacggatacgacattgatgtcttctcttacggcgctccgcgcgtcggtaacagagcgtttgctgaatttttaactgtacaaacaggcggaactctttatcgcatcactcacacaaacgatattgtcccgcgcttacctccgagagaatttggttactcacacagctctcctgaatactggatcaaaagcggtacattggtacctgttactcgaaacgatatcgtcaaaattgaaggaattgacgccaccggcggcaacaaccaaccgaacatccctgacatcccggcacacctttggtacttcggcttaatcggaacatgcctttaaaagctt